European Patent Application EP 4 741 504 A1, published May 13, 2026. Title: 调控AGT表达的dsRNA分子. Applicant: 大睿生物. The sequence listing filed with the application follows.

SEQUENCE LISTING (131 sequences)

SEQ ID NO: 1 - RNA, 19 nt, synthetic construct
  source 1..19: mol_type = other RNA
ctgtttgctgtgtatgata

SEQ ID NO: 2 - RNA, 19 nt, synthetic construct
  source 1..19: mol_type = other RNA
attcctgtttgctgtgtat

SEQ ID NO: 3 - RNA, 19 nt, synthetic construct
  source 1..19: mol_type = other RNA
tttgctgtgtatgatcaaa

SEQ ID NO: 4 - RNA, 19 nt, synthetic construct
  source 1..19: mol_type = other RNA
tgagaagattgacaggttt

SEQ ID NO: 5 - RNA, 19 nt, synthetic construct
  source 1..19: mol_type = other RNA
ctcccaccttttcttctaa

SEQ ID NO: 6 - RNA, 19 nt, synthetic construct
  source 1..19: mol_type = other RNA
tcccaccttttcttctaat

SEQ ID NO: 7 - RNA, 19 nt, synthetic construct
  source 1..19: mol_type = other RNA
cccaccttttcttctaata

SEQ ID NO: 8 - RNA, 19 nt, synthetic construct
  source 1..19: mol_type = other RNA
ttcttctaatgagtcgact

SEQ ID NO: 9 - RNA, 19 nt, synthetic construct
  source 1..19: mol_type = other RNA
tcttctaatgagtcgactt

SEQ ID NO: 10 - RNA, 19 nt, synthetic construct
  source 1..19: mol_type = other RNA
cttctaatgagtcgacttt

SEQ ID NO: 11 - RNA, 19 nt, synthetic construct
  source 1..19: mol_type = other RNA
aagcagccgtttctcctta

SEQ ID NO: 12 - RNA, 19 nt, synthetic construct
  source 1..19: mol_type = other RNA
agccgtttctccttggtct

SEQ ID NO: 13 - RNA, 19 nt, synthetic construct
  source 1..19: mol_type = other RNA
gccgtttctccttggtcta

SEQ ID NO: 14 - RNA, 19 nt, synthetic construct
  source 1..19: mol_type = other RNA
ccgtttctccttggtctaa

SEQ ID NO: 15 - RNA, 19 nt, synthetic construct
  source 1..19: mol_type = other RNA
cgtttctccttggtctaaa

SEQ ID NO: 16 - RNA, 19 nt, synthetic construct
  source 1..19: mol_type = other RNA
gtttctccttggtctaagt

SEQ ID NO: 17 - RNA, 19 nt, synthetic construct
  source 1..19: mol_type = other RNA
ctgcaaaaattgagcaata

SEQ ID NO: 18 - RNA, 19 nt, synthetic construct
  source 1..19: mol_type = other RNA
tcaactggatgaagaaact

SEQ ID NO: 19 - RNA, 19 nt, synthetic construct
  source 1..19: mol_type = other RNA
tctcccaccttttcttcta

SEQ ID NO: 20 - RNA, 19 nt, synthetic construct
  source 1..19: mol_type = other RNA
gtttctccttggtctaaga

SEQ ID NO: 21 - RNA, 21 nt, synthetic construct
  source 1..21: mol_type = other RNA
tatcatacacagcaaacagga

SEQ ID NO: 22 - RNA, 21 nt, synthetic construct
  source 1..21: mol_type = other RNA
atacacagcaaacaggaatgg

SEQ ID NO: 23 - RNA, 21 nt, synthetic construct
  source 1..21: mol_type = other RNA
tttgatcatacacagcaaaca

SEQ ID NO: 24 - RNA, 21 nt, synthetic construct
  source 1..21: mol_type = other RNA
aaacctgtcaatcttctcagc

SEQ ID NO: 25 - RNA, 21 nt, synthetic construct
  source 1..21: mol_type = other RNA
ttagaagaaaaggtgggagac

SEQ ID NO: 26 - RNA, 21 nt, synthetic construct
  source 1..21: mol_type = other RNA
attagaagaaaaggtgggaga

SEQ ID NO: 27 - RNA, 21 nt, synthetic construct
  source 1..21: mol_type = other RNA
tattagaagaaaaggtgggag

SEQ ID NO: 28 - RNA, 21 nt, synthetic construct
  source 1..21: mol_type = other RNA
agtcgactcattagaagaaaa

SEQ ID NO: 29 - RNA, 21 nt, synthetic construct
  source 1..21: mol_type = other RNA
aagtcgactcattagaagaaa

SEQ ID NO: 30 - RNA, 21 nt, synthetic construct
  source 1..21: mol_type = other RNA
aaagtcgactcattagaagaa

SEQ ID NO: 31 - RNA, 21 nt, synthetic construct
  source 1..21: mol_type = other RNA
taaggagaaacggctgctttc

SEQ ID NO: 32 - RNA, 21 nt, synthetic construct
  source 1..21: mol_type = other RNA
agaccaaggagaaacggctgc

SEQ ID NO: 33 - RNA, 21 nt, synthetic construct
  source 1..21: mol_type = other RNA
tagaccaaggagaaacggctg

SEQ ID NO: 34 - RNA, 21 nt, synthetic construct
  source 1..21: mol_type = other RNA
ttagaccaaggagaaacggct

SEQ ID NO: 35 - RNA, 21 nt, synthetic construct
  source 1..21: mol_type = other RNA
tttagaccaaggagaaacggc

SEQ ID NO: 36 - RNA, 21 nt, synthetic construct
  source 1..21: mol_type = other RNA
acttagaccaaggagaaacgg

SEQ ID NO: 37 - RNA, 21 nt, synthetic construct
  source 1..21: mol_type = other RNA
tattgctcaatttttgcaggt

SEQ ID NO: 38 - RNA, 21 nt, synthetic construct
  source 1..21: mol_type = other RNA
agtttcttcatccagttgagg

SEQ ID NO: 39 - RNA, 21 nt, synthetic construct
  source 1..21: mol_type = other RNA
tagaagaaaaggtgggagact

SEQ ID NO: 40 - RNA, 21 nt, synthetic construct
  source 1..21: mol_type = other RNA
tcttagaccaaggagaaacgg

SEQ ID NO: 41 - RNA, 19 nt, synthetic construct
  source 1..19: mol_type = other RNA
ctgtttgctgtgtatgata

SEQ ID NO: 42 - RNA, 19 nt, synthetic construct
  source 1..19: mol_type = other RNA
attcctgtttgctgtgtat

SEQ ID NO: 43 - RNA, 19 nt, synthetic construct
  source 1..19: mol_type = other RNA
tttgctgtgtatgatcaaa

SEQ ID NO: 44 - RNA, 19 nt, synthetic construct
  source 1..19: mol_type = other RNA
tgagaagattgacaggttt

SEQ ID NO: 45 - RNA, 19 nt, synthetic construct
  source 1..19: mol_type = other RNA
ctcccaccttttcttctaa

SEQ ID NO: 46 - RNA, 19 nt, synthetic construct
  source 1..19: mol_type = other RNA
tcccaccttttcttctaat

SEQ ID NO: 47 - RNA, 19 nt, synthetic construct
  source 1..19: mol_type = other RNA
cccaccttttcttctaata

SEQ ID NO: 48 - RNA, 19 nt, synthetic construct
  source 1..19: mol_type = other RNA
ttcttctaatgagtcgact

SEQ ID NO: 49 - RNA, 19 nt, synthetic construct
  source 1..19: mol_type = other RNA
tcttctaatgagtcgactt

SEQ ID NO: 50 - RNA, 19 nt, synthetic construct
  source 1..19: mol_type = other RNA
cttctaatgagtcgacttt

SEQ ID NO: 51 - RNA, 19 nt, synthetic construct
  source 1..19: mol_type = other RNA
aagcagccgtttctcctta

SEQ ID NO: 52 - RNA, 19 nt, synthetic construct
  source 1..19: mol_type = other RNA
agccgtttctccttggtct

SEQ ID NO: 53 - RNA, 19 nt, synthetic construct
  source 1..19: mol_type = other RNA
gccgtttctccttggtcta

SEQ ID NO: 54 - RNA, 19 nt, synthetic construct
  source 1..19: mol_type = other RNA
ccgtttctccttggtctaa

SEQ ID NO: 55 - RNA, 19 nt, synthetic construct
  source 1..19: mol_type = other RNA
cgtttctccttggtctaaa

SEQ ID NO: 56 - RNA, 19 nt, synthetic construct
  source 1..19: mol_type = other RNA
gtttctccttggtctaagt

SEQ ID NO: 57 - RNA, 19 nt, synthetic construct
  source 1..19: mol_type = other RNA
ctgcaaaaattgagcaata

SEQ ID NO: 58 - RNA, 19 nt, synthetic construct
  source 1..19: mol_type = other RNA
tcaactggatgaagaaact

SEQ ID NO: 59 - RNA, 19 nt, synthetic construct
  source 1..19: mol_type = other RNA
tctcccaccttttcttcta

SEQ ID NO: 60 - RNA, 19 nt, synthetic construct
  source 1..19: mol_type = other RNA
ctgtttgctgtgtatgata

SEQ ID NO: 61 - RNA, 19 nt, synthetic construct
  source 1..19: mol_type = other RNA
attcctgtttgctgtgtat

SEQ ID NO: 62 - RNA, 19 nt, synthetic construct
  source 1..19: mol_type = other RNA
tttgctgtgtatgatcaaa

SEQ ID NO: 63 - RNA, 19 nt, synthetic construct
  source 1..19: mol_type = other RNA
tgagaagattgacaggttt

SEQ ID NO: 64 - RNA, 19 nt, synthetic construct
  source 1..19: mol_type = other RNA
ctcccaccttttcttctaa

SEQ ID NO: 65 - RNA, 19 nt, synthetic construct
  source 1..19: mol_type = other RNA
tcccaccttttcttctaat

SEQ ID NO: 66 - RNA, 19 nt, synthetic construct
  source 1..19: mol_type = other RNA
cccaccttttcttctaata

SEQ ID NO: 67 - RNA, 19 nt, synthetic construct
  source 1..19: mol_type = other RNA
ttcttctaatgagtcgact

SEQ ID NO: 68 - RNA, 19 nt, synthetic construct
  source 1..19: mol_type = other RNA
tcttctaatgagtcgactt

SEQ ID NO: 69 - RNA, 19 nt, synthetic construct
  source 1..19: mol_type = other RNA
cttctaatgagtcgacttt

SEQ ID NO: 70 - RNA, 19 nt, synthetic construct
  source 1..19: mol_type = other RNA
aagcagccgtttctcctta

SEQ ID NO: 71 - RNA, 19 nt, synthetic construct
  source 1..19: mol_type = other RNA
agccgtttctccttggtct

SEQ ID NO: 72 - RNA, 19 nt, synthetic construct
  source 1..19: mol_type = other RNA
gccgtttctccttggtcta

SEQ ID NO: 73 - RNA, 19 nt, synthetic construct
  source 1..19: mol_type = other RNA
ccgtttctccttggtctaa

SEQ ID NO: 74 - RNA, 19 nt, synthetic construct
  source 1..19: mol_type = other RNA
cgtttctccttggtctaaa

SEQ ID NO: 75 - RNA, 19 nt, synthetic construct
  source 1..19: mol_type = other RNA
gtttctccttggtctaagt

SEQ ID NO: 76 - RNA, 19 nt, synthetic construct
  source 1..19: mol_type = other RNA
ctgcaaaaattgagcaata

SEQ ID NO: 77 - RNA, 19 nt, synthetic construct
  source 1..19: mol_type = other RNA
tcaactggatgaagaaact

SEQ ID NO: 78 - RNA, 19 nt, synthetic construct
  source 1..19: mol_type = other RNA
tctcccaccttttcttcta

SEQ ID NO: 79 - RNA, 19 nt, synthetic construct
  source 1..19: mol_type = other RNA
gtttctccttggtctaaga

SEQ ID NO: 80 - RNA, 21 nt, synthetic construct
  source 1..21: mol_type = other RNA
gtcatccacaatgagagtaca

SEQ ID NO: 81 - RNA, 21 nt, synthetic construct
  source 1..21: mol_type = other RNA
tatcatacacagcaaacagga

SEQ ID NO: 82 - RNA, 21 nt, synthetic construct
  source 1..21: mol_type = other RNA
atacacagcaaacaggaatgg

SEQ ID NO: 83 - RNA, 21 nt, synthetic construct
  source 1..21: mol_type = other RNA
tttgatcatacacagcaaaca

SEQ ID NO: 84 - RNA, 21 nt, synthetic construct
  source 1..21: mol_type = other RNA
aaacctgtcaatcttctcagc

SEQ ID NO: 85 - RNA, 21 nt, synthetic construct
  source 1..21: mol_type = other RNA
ttagaagaaaaggtgggagac

SEQ ID NO: 86 - RNA, 21 nt, synthetic construct
  source 1..21: mol_type = other RNA
attagaagaaaaggtgggaga

SEQ ID NO: 87 - RNA, 21 nt, synthetic construct
  source 1..21: mol_type = other RNA
tattagaagaaaaggtgggag

SEQ ID NO: 88 - RNA, 21 nt, synthetic construct
  source 1..21: mol_type = other RNA
agtcgactcattagaagaaaa

SEQ ID NO: 89 - RNA, 21 nt, synthetic construct
  source 1..21: mol_type = other RNA
aagtcgactcattagaagaaa

SEQ ID NO: 90 - RNA, 21 nt, synthetic construct
  source 1..21: mol_type = other RNA
aaagtcgactcattagaagaa

SEQ ID NO: 91 - RNA, 21 nt, synthetic construct
  source 1..21: mol_type = other RNA
taaggagaaacggctgctttc

SEQ ID NO: 92 - RNA, 21 nt, synthetic construct
  source 1..21: mol_type = other RNA
agaccaaggagaaacggctgc

SEQ ID NO: 93 - RNA, 21 nt, synthetic construct
  source 1..21: mol_type = other RNA
tagaccaaggagaaacggctg

SEQ ID NO: 94 - RNA, 21 nt, synthetic construct
  source 1..21: mol_type = other RNA
ttagaccaaggagaaacggct

SEQ ID NO: 95 - RNA, 21 nt, synthetic construct
  source 1..21: mol_type = other RNA
tttagaccaaggagaaacggc

SEQ ID NO: 96 - RNA, 21 nt, synthetic construct
  source 1..21: mol_type = other RNA
acttagaccaaggagaaacgg

SEQ ID NO: 97 - RNA, 21 nt, synthetic construct
  source 1..21: mol_type = other RNA
tattgctcaatttttgcaggt

SEQ ID NO: 98 - RNA, 21 nt, synthetic construct
  source 1..21: mol_type = other RNA
agtttcttcatccagttgagg

SEQ ID NO: 99 - RNA, 21 nt, synthetic construct
  source 1..21: mol_type = other RNA
tagaagaaaaggtgggagact

SEQ ID NO: 100 - RNA, 21 nt, synthetic construct
  source 1..21: mol_type = other RNA
tagaccaaggagaaacggctg

SEQ ID NO: 101 - RNA, 21 nt, synthetic construct
  source 1..21: mol_type = other RNA
  modified_base 7: mod_base = OTHER; note = a is (Agn)
tagaccaaggagaaacggctg

SEQ ID NO: 102 - RNA, 21 nt, synthetic construct
  source 1..21: mol_type = other RNA
  modified_base 1: mod_base = OTHER; note = t is (SCP-U)
  modified_base 2: mod_base = OTHER; note = a is dA
  modified_base 5: mod_base = OTHER; note = c is dC
  modified_base 7: mod_base = OTHER; note = a is dA
  modified_base 12: mod_base = OTHER; note = g is dG
tagaccaaggagaaacggctg

SEQ ID NO: 103 - RNA, 21 nt, synthetic construct
  source 1..21: mol_type = other RNA
  modified_base 1: mod_base = OTHER; note = t is (SCP-U)
  modified_base 7: mod_base = OTHER; note = a is (Agn)
tagaccaaggagaaacggctg

SEQ ID NO: 104 - RNA, 21 nt, synthetic construct
  source 1..21: mol_type = other RNA
  modified_base 1: mod_base = OTHER; note = t is (SCP-U)
  modified_base 7: mod_base = OTHER; note = a is (Agn)
tcttagaccaaggagaaacgg

SEQ ID NO: 105 - RNA, 21 nt, synthetic construct
  source 1..21: mol_type = other RNA
  modified_base 1: mod_base = OTHER; note = t is (SCP-U)
  modified_base 2: mod_base = OTHER; note = c is dC
  modified_base 5: mod_base = OTHER; note = a is dA
  modified_base 7: mod_base = OTHER; note = a is dA
  modified_base 12: mod_base = OTHER; note = g is dG
tcttagaccaaggagaaacgg

SEQ ID NO: 106 - RNA, 23 nt, synthetic construct
  source 1..23: mol_type = other RNA
  modified_base 6: mod_base = OTHER; note = t is (Tgn)
tgtactctcattgtggatgacga

SEQ ID NO: 107 - DNA, 20 bp, synthetic construct
  source 1..20: mol_type = other DNA
acgtggacatccgcaaagac

SEQ ID NO: 108 - DNA, 20 bp, synthetic construct
  source 1..20: mol_type = other DNA
tcttcattgtgctgggtgcc

SEQ ID NO: 109 - DNA, 25 bp, synthetic construct
  source 1..25: mol_type = other DNA
aacacagtgctgtctggcggcacca

SEQ ID NO: 110 - DNA, 19 bp, synthetic construct
  source 1..19: mol_type = other DNA
tgtgagcagctggcaaagg

SEQ ID NO: 111 - DNA, 21 bp, synthetic construct
  source 1..21: mol_type = other DNA
gatgtcttggcctgaattgga

SEQ ID NO: 112 - DNA, 14 bp, synthetic construct
  source 1..14: mol_type = other DNA
caatgccgggaagc

SEQ ID NO: 113 - RNA, 19 nt, synthetic construct
  source 1..19: mol_type = other RNA
ctgtttgctgtgtatgata

SEQ ID NO: 114 - RNA, 19 nt, synthetic construct
  source 1..19: mol_type = other RNA
attcctgtttgctgtgtat

SEQ ID NO: 115 - RNA, 19 nt, synthetic construct
  source 1..19: mol_type = other RNA
tttgctgtgtatgatcaaa

SEQ ID NO: 116 - RNA, 19 nt, synthetic construct
  source 1..19: mol_type = other RNA
tgagaagattgacaggttt

SEQ ID NO: 117 - RNA, 19 nt, synthetic construct
  source 1..19: mol_type = other RNA
ctcccaccttttcttctaa

SEQ ID NO: 118 - RNA, 19 nt, synthetic construct
  source 1..19: mol_type = other RNA
tcccaccttttcttctaat

SEQ ID NO: 119 - RNA, 19 nt, synthetic construct
  source 1..19: mol_type = other RNA
cccaccttttcttctaata

SEQ ID NO: 120 - RNA, 19 nt, synthetic construct
  source 1..19: mol_type = other RNA
ttcttctaatgagtcgact

SEQ ID NO: 121 - RNA, 19 nt, synthetic construct
  source 1..19: mol_type = other RNA
tcttctaatgagtcgactt

SEQ ID NO: 122 - RNA, 19 nt, synthetic construct
  source 1..19: mol_type = other RNA
cttctaatgagtcgacttt

SEQ ID NO: 123 - RNA, 19 nt, synthetic construct
  source 1..19: mol_type = other RNA
aagcagccgtttctcctta

SEQ ID NO: 124 - RNA, 19 nt, synthetic construct
  source 1..19: mol_type = other RNA
agccgtttctccttggtct

SEQ ID NO: 125 - RNA, 19 nt, synthetic construct
  source 1..19: mol_type = other RNA
gccgtttctccttggtcta

SEQ ID NO: 126 - RNA, 19 nt, synthetic construct
  source 1..19: mol_type = other RNA
ccgtttctccttggtctaa

SEQ ID NO: 127 - RNA, 19 nt, synthetic construct
  source 1..19: mol_type = other RNA
cgtttctccttggtctaaa

SEQ ID NO: 128 - RNA, 19 nt, synthetic construct
  source 1..19: mol_type = other RNA
gtttctccttggtctaagt

SEQ ID NO: 129 - RNA, 19 nt, synthetic construct
  source 1..19: mol_type = other RNA
ctgcaaaaattgagcaata

SEQ ID NO: 130 - RNA, 19 nt, synthetic construct
  source 1..19: mol_type = other RNA
tcaactggatgaagaaact

SEQ ID NO: 131 - RNA, 19 nt, synthetic construct
  source 1..19: mol_type = other RNA
tctcccaccttttcttcta